European Patent Application EP 4 589 014 A2, published July 23, 2025. Title: Immunotherapy Methods for Patients Whose Tumors Carry a High Passenger Gene Mutation Burden. Applicant: Regeneron Pharmaceuticals, Inc. The sequence listing filed with the application follows.

SEQUENCE LISTING (217 sequences)

SEQ ID NO: 1 - protein, 121 aa, synthetic construct
  REGION 1..121: note = synthetic construct; antigen binding domain
EVQLLESGGGLVQPGGSLRLSCSASGFTFSSYTMNWVRQAPGKGLEWVSGISDTGGNTYYTDSVKGRFTVSRDNSKNTLSLQMNSLRAEDTAVYYCAKDQGGSYPYYFHYWGQGSLVTVSS

SEQ ID NO: 2 - protein, 108 aa, synthetic construct
  REGION 1..108: note = synthetic construct; antigen binding domain
DIQMTQSPSSLSASVGDRVTITCRASQSISSYLIWYQQKPGTAPKFLIYAASSLQSGVPSRFSGCGSGTDFTLTISSLQPEDFATYYCQQSYSTPPITFGQGTRLEIK

SEQ ID NO: 3 - protein, 122 aa, synthetic construct
  REGION 1..122: note = synthetic construct; antigen binding domain
EVQLVESGGGLVQPGGSLRLSCAASGFTVSNNYMSWVRQAPGKGLEWVSVIYSGGFTYYTDSVKGRFTISRHNSKNTLYLQMNSLRAEDTAVYYCARYYYDTSDYWTFFDYWGQGTLVTVSS

SEQ ID NO: 4 - protein, 107 aa, synthetic construct
  REGION 1..107: note = synthetic construct; antigen binding domain
EIVMTQSPATLSVSPGERATLSCRASQSVSSNLAWYQQKPGQAPRLLIYGASTRATGIPARFSGSGSGTEFTLTISSLQSGDFAVYYCQQYNNWPLTFGGGTKVEIN

SEQ ID NO: 5 - protein, 122 aa, synthetic construct; identical to SEQ ID NO: 3
  REGION 1..122: note = synthetic construct; antigen binding domain

SEQ ID NO: 6 - protein, 107 aa, synthetic construct; identical to SEQ ID NO: 4
  REGION 1..107: note = synthetic construct; antigen binding domain

SEQ ID NO: 7 - protein, 119 aa, synthetic construct
  REGION 1..119: note = synthetic construct; antigen binding domain
QVQLVESGGGVVQSGRSLRLSCAASGFTFSSYGMHWVRQAPGKGLEWVAVIWYDGSNIYYSDSVKGRFTISRANSKNTLYLQMNSLRAEDTAVYYCARPGHWNYFFEYWGQGTLVTVSS

SEQ ID NO: 8 - protein, 108 aa, synthetic construct
  REGION 1..108: note = synthetic construct; antigen binding domain
DIQMTQSPSSLSASVGDRVTITCRASQSINNYLNWYQQKPGKAPKLLIYTASSLQSGVPSRFSGSGSGTDFTLTISSLQPEDFATYYCQQSYSTPPLTFGQGTQLEIK

SEQ ID NO: 9 - protein, 122 aa, synthetic construct
  REGION 1..122: note = synthetic construct; antigen binding domain
EVQLVESGGGLVQPGGSLRLSCGASGFTFRNYDMHWVRQITGKGLEWVSAIGSAGDTYYPDSVKGRFTISRENAKNSLYLQMNSLRVGDTAVYYCTRDIHCSSTRCYGMDVWGQGTTVTVSS

SEQ ID NO: 10 - protein, 108 aa, synthetic construct
  REGION 1..108: note = synthetic construct; antigen binding domain
DIQMTQSPSSLSASVGDRVTITCRASQSISNYLNWYQQKPGKAPKLLIYAASSLQSGVPSRFSGSGSGTDFTLTISSLQPEDFATYYCQQSYSTPPITFGQGTRLEIK

SEQ ID NO: 11 - protein, 130 aa, synthetic construct
  REGION 1..130: note = synthetic construct; antigen binding domain
EVQLVESGGGLVKPGGSLRLSCAASGFKFSNEWMSWVRQAPGKGLEWVGRIKSKTDGGTTDYAAPVKGRFTISRDDSKNTLYLQMNSLKTEDTAVYYCTTDQDFWSGYYTGADYYGMDVWGQGTMVTVSS

SEQ ID NO: 12 - protein, 108 aa, synthetic construct
  REGION 1..108: note = synthetic construct; antigen binding domain
DIQMTQSPSSLSASVGDRVTITCRASQSISSYLNWYQQKPGKAPKLLIYAASSLQSGVPSRFSGSGSGTDFTLTISSLQPEDFATYYCQQSYSTPPITFGQGTRLEIK

SEQ ID NO: 13 - protein, 116 aa, synthetic construct
  REGION 1..116: note = synthetic construct; antigen binding domain
QMQLQQWGAGLLKPSETLSLTCVVYGGSLNGYYWSWIRQSPGKGLEWIGEIDHSGSTNYNPSLKNRVTMSVDTSKIQFSLKLTSVTVADTAVYYCAREGLLPFDYWGQGTLVTVSS

SEQ ID NO: 14 - protein, 108 aa, synthetic construct
  REGION 1..108: note = synthetic construct; antigen binding domain
EIVLTQSPGTLSLSPGERVTLSCRASQSVYSNYLAWYQQNPGQAPRLLIYAASNRATGIPDRFSGSGSGTDFTLTISRLEPEDFAVYYCHQYATSPWTFGQGTKVEIK

SEQ ID NO: 15 - protein, 123 aa, synthetic construct
  REGION 1..123: note = synthetic construct; antigen binding domain
QLQLQESGPDLVKPSDTLSLTCTVSDDSISSTTYYWAWIRQPPGKGLEWIGSMSYNGNNYYNPSLKSRVAISAGTSQKQFSLKLTSVTAADTAVYHCARHLGYNGNWYPFDFWGQGILVTVSS

SEQ ID NO: 16 - protein, 108 aa, synthetic construct
  REGION 1..108: note = synthetic construct; antigen binding domain
EIVLTQSPGTLSLSPGERATLSCRASQSVSSSYLAWYQQKPGQAPRLLIYGASSRTTGIPDRFSGSGSGTDFTLTISRLEPEDFAVYYCQQYGSSPWTFGQGTKVEIK

SEQ ID NO: 17 - protein, 122 aa, synthetic construct
  REGION 1..122: note = synthetic construct; antigen binding domain
EVQVVESGGGLVEPGRSLRLSCKASGFTFDDYAMHWVRQTPGKALEWVSGINWSGNNIGYADSVKGRFTISKDDAKNSLYLQMNSLRPEDTALYYCTKDISITGTLDAFDVWGQGTMVTVSS

SEQ ID NO: 18 - protein, 107 aa, synthetic construct
  REGION 1..107: note = synthetic construct; antigen binding domain
DIQMTQSPISVSASVGDRVTITCRASQGISNWLAWYQQKPGIAPKLLIYSASSLQSGVPSRFRGSGSGTDFTLTIGSLQPEDFATYYCQQAHSFPLTFGGGTKVEIK

SEQ ID NO: 19 - protein, 116 aa, synthetic construct
  REGION 1..116: note = synthetic construct; antigen binding domain
QVQLVESGGGVVQPGRSLRLSCAASGFTFSSYGMHWVRQAPGKGLEWVAIIWSDGDSEYNLDSVKGRFTISRDNSKNTLYLQMNSLRVEDSAVYYCARDRDLEDIWGQGTMVTVSS

SEQ ID NO: 20 - protein, 107 aa, synthetic construct
  REGION 1..107: note = synthetic construct; antigen binding domain
DIQMTQSPSSLSASVGDRVTITCRASQGIRNDLGWYQQKPGKAPKRLIYAASNLQSGVPSRFSGSGSGTEFTLTISSLQPEDFATYYCLQHNSYPLTFGGGTKVEIK

SEQ ID NO: 21 - protein, 117 aa, synthetic construct [sequence omitted]

SEQ ID NO: 22 - protein, 107 aa, synthetic construct [sequence omitted]

SEQ ID NO: 23 - protein, 121 aa, synthetic construct
  REGION 1..121: note = synthetic construct; antigen binding domain
EVQLVESGGGVVRPGGSLRLSCAASGFTFDDYGMSWVRQVPGKGLEWVSGISWNDGKTVYAESVKGRFIISRDNAKNSLYLEMNSLRAEDTALYYCARDWQYLIERYFDYWGQGTLVTVSS

SEQ ID NO: 24 - protein, 108 aa, synthetic construct
  REGION 1..108: note = synthetic construct; antigen binding domain
EIVLTQSPGTLSLSPGERATLSCRASQSVSSSYLAWYQQKPGQAPRLLIYGASSRATGIPDRFSGSGSGTDFTLTISRLEPEDFAVYYCQQYGSSPWTFGQGTKVEIK

SEQ ID NO: 25 - protein, 121 aa, synthetic construct
  REGION 1..121: note = synthetic construct; antigen binding domain
EVQLVESGGGVVRPGGSLRLSCTASGFTFDDYGMSWVRQAPGKGLEWISGIGWTGGRSSYADSVRGRFTISRDNAKNSLYLQMNSLGAEDTALYYCARDRQWLVQWYFDYWGQGTLVTVSS

SEQ ID NO: 26 - protein, 108 aa, synthetic construct; identical to SEQ ID NO: 12
  REGION 1..108: note = synthetic construct; antigen binding domain

SEQ ID NO: 27 - protein, 121 aa, synthetic construct
  REGION 1..121: note = synthetic construct; antigen binding domain
EVQLVESGGRVVRPGGSLRLSCAASGFTFDDYGMSWVRQLPGKGLEWVAGISWNDGKTVYAESVKGRFIISRDNAKNSLHLEMNSLRAEDTALYYCARDWQYLIDRYFDFWGQGTLVTVSS

SEQ ID NO: 28 - protein, 121 aa, synthetic construct
  REGION 1..121: note = synthetic construct; antigen binding domain
EVQLVESGGGLVQPGGSLRLSCAASGFTFDDYAMHWVRQAPGKGLEWVSGIGWSSGSIGYADSVKGRFTISRDNAKNSLYLQMDSLRPEDSALYYCAKAYTFMITLYFDYWGQGTLVTVSS

SEQ ID NO: 29 - protein, 121 aa, synthetic construct
  REGION 1..121: note = synthetic construct; antigen binding domain
EVQLVESGGGLVQPGRSLRLSCAASGFTFDDYDMHWVRQAPGKGLEWVSGSGWNRGSLGYADSVKGRFTISRDNAKKSLYLQMNSVRVEDTALYYCAKGFVVVSAAYFDYWGQGTLVTVSS

SEQ ID NO: 30 - protein, 121 aa, synthetic construct
  REGION 1..121: note = synthetic construct; antigen binding domain
QVQLVQSGAEVKRPGSSVKVSCKVSGVTFRNFAIIWVRQAPGQGLEWMGGIIPFFSAANYAQSFQGRVTITPDESTSTAFMELASLRSEDTAVYYCAREGERGHTYGFDYWGQGTLVTVSS

SEQ ID NO: 31 - protein, 121 aa, synthetic construct
  REGION 1..121: note = synthetic construct; antigen binding domain
EVQLVESGGGLVQSGRSLRLSCAASGFTFDDYAMHWVRQPPGKGLEWVSGINWNRGRTGYADSVKGRFTISRDNAKNSLYLQMNDLRVEDTALYYCAKAEQWLDEGYFDYWGQGTLVTVSS

SEQ ID NO: 32 - protein, 121 aa, synthetic construct
  REGION 1..121: note = synthetic construct; antigen binding domain
EVQLVESGGGLVQRGGSLRLSCAASGFSFSSYAMNWVRQAPGKGLEWVSTISDSGGSTYYADSVKGRFTISRDNSKNTLSLQMNSLRAEDTAVYYCAKDQGGSYPYYFHYWGQGTLVTVSS

SEQ ID NO: 33 - protein, 121 aa, synthetic construct
  REGION 1..121: note = synthetic construct; antigen binding domain
EVQLVESGGGLVQPGRSLRLSCAASGFTFEDYAMHWVRQAPGKGLEWVSGIGWSNVKIGYADSVKGRFTISRDNVRNSLYLQMNSLRTEDTAFYYCVKAYTSMLTLYFDYWGQGTLVTVSS

SEQ ID NO: 34 - protein, 118 aa, synthetic construct
  REGION 1..118: note = synthetic construct; antigen binding domain
QVQLVQSGAEVKRPGASVKVSCKASGYTFTSFYMYWVRQAPGQGLEWMGIINPSDGSTSNAQKFQGRVTMTRDTSTSTVYMELSSLRSEDTAVYYCARRVAGDIFDIWGQGTMVTVSS

SEQ ID NO: 35 - protein, 119 aa, synthetic construct
  REGION 1..119: note = synthetic construct; antigen binding domain
QVQLQESGPGLVKPSETLSLTCTVSGGSISSYHWNWIRQSPGKGLEWIGYIYYIGSTDYNPSLESRVTISVDTSKNQFSLKLSSVTAADTAVYYCARVPVGATGASDVWGQGTMVTVSS

SEQ ID NO: 36 - protein, 121 aa, synthetic construct
  REGION 1..121: note = synthetic construct; antigen binding domain
EVQLVESGGSVVRPGGSLRLSCVVSGFTFEDYGLSWVRQIPGKGLEWVSGISWTGGNTGYADSVKGRFTISRDNAKNSLYLQMNSLRAEDTALYHCTRDRQWLMQWYFDYWGQGTLVTVSS

SEQ ID NO: 37 - protein, 119 aa, synthetic construct
  REGION 1..119: note = synthetic construct; antigen binding domain
QVQLVESGGGVVQPGRSLRLSCSASGFTFSAYAMHWVRQAPGKGLEWVAAISYGGSDKYYADSVKGRFTISRDNSKNTLYLQMNSLRTDDTAVYYCAKSAHWNFFFDYWGQGTLVTVSS

SEQ ID NO: 38 - protein, 121 aa, synthetic construct
  REGION 1..121: note = synthetic construct; antigen binding domain
EVQLVESGGGLVQPGRSLRLSCVASGFALHDYAMHWVRQVPGKGLEWVSSISWNSGVIGYADSLKGRFTISRDNAKNSLYLQMNSLRAEDTALYYCAKGSGSYYVSWFDPWGQGTLVTVSS

SEQ ID NO: 39 - protein, 123 aa, synthetic construct
  REGION 1..123: note = synthetic construct; antigen binding domain
QLQLQESGPGLVQPSETLSLTCTVSGDSISSTAYHWDWIRQPPGKGLEWIGTITYNGNTYFNPSLKSRVTISVDTSKNQFSLKLLSMTAAETAVFYCARHLGYNSDFFPFDFWGQGTLVTVSS

SEQ ID NO: 40 - protein, 119 aa, synthetic construct
  REGION 1..119: note = synthetic construct; antigen binding domain
EVQLVESGGGLVRPGGSLRLSCAASGFTFSTYAMAWVRQTPGKGLEGVSAIGGSGDSTYYVDSVKGRFTISRDNSKSTLFLQMNSLRAEDTAVYYCVKVRNYDGSFDIWGQGTMVTVSS

SEQ ID NO: 41 - protein, 124 aa, synthetic construct
  REGION 1..124: note = synthetic construct; antigen binding domain
EVQLLESGGGLVQPGGSLRLSCVASGFTFSTYAMSWVRQAPGMGLEWVSSISGSGRNTYYADSVKGRFTISRDNSKNTLFLQMNSLRAEDTAVYYCAKESVTGTSSYYYGVDVWGQGTTVTVSS

SEQ ID NO: 42 - protein, 107 aa, synthetic construct
  REGION 1..107: note = synthetic construct; antigen binding domain
DIQMTQSPSSLSASVGDRVTITCRASQSISSYLNWYHQKPGKAPKLLIYAASSLQNGVPSRFSGSGSGTDFTLTISSLQPEDFASYYCQQSYRTPLTFGGGTKVEIK

SEQ ID NO: 43 - protein, 128 aa, synthetic construct
  REGION 1..128: note = synthetic construct; antigen binding domain
QVQLEESGGGVVQPGRSLRLSCAASGFTFSWYGMHWVRQAPGKGLEWVALIWYDGTNKKYGDSVKGRFTISRDNSKNTVYLQMNSLRAEDTAVYYCARDCGHSGNDRGTYYYYYGMDVWGQGTTVTVS

SEQ ID NO: 44 - protein, 108 aa, synthetic construct; identical to SEQ ID NO: 12
  REGION 1..108: note = synthetic construct; antigen binding domain

SEQ ID NO: 45 - protein, 119 aa, synthetic construct
  REGION 1..119: note = synthetic construct; antigen binding domain
QVQLQQWGAGLLKPSETLSLTCAVYGGSFSGYYWNWIRQPPGKGLEWVGEISHRGTTNYNPSLKSRVTISLDTSKNQFSLKLTSVTAADTAVYYCSRDEELEFRFFDYWGQGTLVTVSS

SEQ ID NO: 46 - protein, 107 aa, synthetic construct
  REGION 1..107: note = synthetic construct; antigen binding domain
EIVLTQSPATLSLSPGERATLSCRASQSVSSYLAWYQQKPGQAPRLLVYGASNRATGIPARFSGSGSGTDFTLTISSLEPEDFAFYYCQQRSNWPLTFGGGTKVEIK

SEQ ID NO: 47 - protein, 119 aa, synthetic construct
  REGION 1..119: note = synthetic construct; antigen binding domain
QLQLQESGPGLVKPSETLSLTCTVSGDSIISNSYYWGWIRQPPGKGLEWIGNFFYTGATYYNPSLKSRVTISADTSKNQFSLKLSSVTAADTALYYCASYNRNYRFDPWGQGTLVTVSS

SEQ ID NO: 48 - protein, 108 aa, synthetic construct
  REGION 1..108: note = synthetic construct; antigen binding domain
DIQMTQSPSSLSASVGDRVTITCRASQSISSYLNWYQQKPGKAPKLLIYAASSLQSGVPSRFSGSGSGTDFTLTISSLQPEDFATYFCQQSYSTPPITFGQGTRLEIK

SEQ ID NO: 49 - protein, 127 aa, synthetic construct
  REGION 1..127: note = synthetic construct; antigen binding domain
QVQLQQWGAGLLKPSETLSLTCAVYGGSFSTYYWSWIRQPPGKGLEWIGEINHSGNADYNPSLKSRVSISVDTSKNQFSLRLSSVTAADTAIYYCARAGYCSSPTCYSYYYFGMDVWGQGTTVTVSS

SEQ ID NO: 50 - protein, 108 aa, synthetic construct
  REGION 1..108: note = synthetic construct; antigen binding domain
EIVLTQSPGTLSLSLGERATLSCRASQSVISSFLAWYQQKPGQAPRLLIYGASSRATGFPDRFSGSGSGTDFTLTIRRLEPEDFAVYYCQQYGNSPWTFGQGTKVEIK

SEQ ID NO: 51 - protein, 129 aa, synthetic construct
  REGION 1..129: note = synthetic construct; antigen binding domain
QVTLKESGPVLVKPTETLTLTCTVSGFSLSNAGMGVSWVRQPPGKALEWLAHIFSNDEKSYSTSLRTRLTISKDTSKSQVVLTVTNLDPVDTATYFCARIPEFTSSSWALYYFYGMDVWGQGTTVTVSS

SEQ ID NO: 52 - protein, 108 aa, synthetic construct
  REGION 1..108: note = synthetic construct; antigen binding domain
EIVLTQSPGTLSLSPGESATLSCRASQSITSTYFAWYQQKPGQAPRLLIYATSSRATGVPDRFSGSGSGTDFTLTISRLEPDDFAVYYCQQYGRSPWTFGQGTKVEVK

SEQ ID NO: 53 - protein, 121 aa, synthetic construct
  REGION 1..121: note = synthetic construct; antigen binding domain
QVQLVQSGAEVKKPGASVKVSCKASGYTFTSYGISWVRQAPGQGLEWMGWISAYNDNTNYAQKLQGRVTMTADTSTNTAYMELRSLRSDDTAIYYCVRWNWGSVYWYFDLWGRGTLVTVSS

SEQ ID NO: 54 - protein, 108 aa, synthetic construct
  REGION 1..108: note = synthetic construct; antigen binding domain
EIVLTQSPGTLSLSPGERATLSCRASQIISSSYFAWYQQKPGQAPRLLIYGASSRATGIPDRFSGSVSGTDFTLTISRLEPEDFAMYFCQQYGNSPWTFGQGTKVEIK

SEQ ID NO: 55 - protein, 117 aa, synthetic construct
  REGION 1..117: note = synthetic construct; antigen binding domain
QITLKESGPTLVKPTQTLTLTCTFSGFSLNTHRVGVGWIRQPPGKALEWLALIYGNDVKNYSPSLETRLTIAKDTSKNQVVLTMTNMDPVDTATYFCSYITGEGMYWGQGTLVTVSS

SEQ ID NO: 56 - protein, 111 aa, synthetic construct
  REGION 1..111: note = synthetic construct; antigen binding domain
DVVMTQSPLSLSVTLGQPASISCRSSQNLMYSDGNTYLNWFHQRPGQSPRRLIYKVSNRDSGVPDRFSGSGSGTDFTLKISRVEAEDVGVYYCMQGTHWYTFGQGTKLEIK

SEQ ID NO: 57 - protein, 119 aa, synthetic construct
  REGION 1..119: note = synthetic construct; antigen binding domain
QVQLQQWGAGLLKPSETLSLTCAVYGGSFSGYYWSWIRQPPGKGLEWIGEINHRGNTNYNPSLKSRVTISLDTSKKQFSLNLSSVTAADTAMYYCTRDEEQELRFLDYWGQGTLVTVSS

SEQ ID NO: 58 - protein, 107 aa, synthetic construct
  REGION 1..107: note = synthetic construct; antigen binding domain
EIVLTQSPATLSLSPGERATLSCRASQDISTYLAWYQQRAGQAPRLLIYGASNRATGIPARFSGSGSGTDFTLTISSLEPEDFAFYYCQQRSNWPLTFGGGTEVEIK

SEQ ID NO: 59 - protein, 122 aa, synthetic construct
  REGION 1..122: note = synthetic construct; antigen binding domain
QVQLQQWGAGLLKPSETLSLTCVVHGGSFSGYYWNWIRQPPGKGLEWIGEINHRGNTNYNPSLKSRVTVSEDTSKNQFSLKLSSLTAADTAVYYCVRGEDYDFWSDYYNDYWGQGTLVTVSS

SEQ ID NO: 60 - protein, 107 aa, synthetic construct
  REGION 1..107: note = synthetic construct; antigen binding domain
EIVLTQSPATLSLSPGERATLSCRASQTISSYLAWHQQKPGQAPRLLIYDASKRATGIPARFSGSGSGTDFTLTITSLEPEDFAVYYCQQRSNWPLTFGGGTKVEIK

SEQ ID NO: 61 - protein, 124 aa, synthetic construct
  REGION 1..124: note = synthetic construct; antigen binding domain
QVQLQQWGAGLLPPSETLSLICAVYGGSFSGYYWSWIRQPPGKGLEWIGEINHRGSTNYNPSLKSRATISVDTSKNQFSLKLSSVTAADTAVYYCSRGEDYYDSSGYSYYFDYWGQGTLVTVSS

SEQ ID NO: 62 - protein, 107 aa, synthetic construct
  REGION 1..107: note = synthetic construct; antigen binding domain
EIVLTQSPATLSLSPGERATLSCRASQSVSSYLAWYQQKPGQAPRLLIYDASNRATGIPARFSGSGSGTDFTLTISSLEPEDFAVYYCQQRSNWPLTFGGGTKVEIK

SEQ ID NO: 63 - protein, 122 aa, synthetic construct
  REGION 1..122: note = synthetic construct; antigen binding domain
QVQLQQWGAGLLRPSETLSLTCAVYGGSFSGYYWNWIRQSPGTGLEWIGEINHRGNINFNPSLKSRVTISEDTSKNQFSLRLNSVTAADTAVYYCARGEDYDIWSGYYREYWGQGTLVTVSS

SEQ ID NO: 64 - protein, 107 aa, synthetic construct
  REGION 1..107: note = synthetic construct; antigen binding domain
EIVLTQSPATLSLSPGERATLSCRASQSVSSYLAWYQQKPGQAPRLLIYDASKRATGIPARFSGSGSGTDFTLTISSLEPEDFAVYYCQQRSNWPLAFGGGTKVEIK

SEQ ID NO: 65 - protein, 119 aa, synthetic construct
  REGION 1..119: note = synthetic construct; antigen binding domain
QVQLQQWGAGLLKPSETLSLTCAVYGGSFSEFYWNWIRQPPEKGLEWIGEINHRGNTNYNPSLKSRVTISVDMSKNQFSLQLNSVTVADTALYYCAFGYDFRSSYEDVWGQGTTVTVSS

SEQ ID NO: 66 - protein, 107 aa, synthetic construct
  REGION 1..107: note = synthetic construct; antigen binding domain
EIVLTQSPATLSLSPGERATLSCRASQDISTYLAWHQQKPGQPPRLLIYGSSNRATGIPARFSGSGSGTDFTLTISSLEPEDFAVYYCQQRSNWPLTFGGGTKVEIK

SEQ ID NO: 67 - protein, 124 aa, synthetic construct
  REGION 1..124: note = synthetic construct; antigen binding domain
EVQLLESGGGLVQPGGSLRLSCAASGFTFRSYAMSWVRQAPGKGLEWVSVISGGGGRTYYTDSVKGRFTISRDNSKSMLYLQMNSLRAEDTAIYYCAKERVTGIDHYYYGVDVWGQGTTVTVSS

SEQ ID NO: 68 - protein, 107 aa, synthetic construct
  REGION 1..107: note = synthetic construct; antigen binding domain
DIQMTQSPSSLSASVGDRVTITCRASQSISSYLNWYQQKPGKAPKLLIYATSSLQSGVPSRFSGSASGTDFTLAISSLQPEDFATYYCQQSYTTPLTFGGGTKVEIK

SEQ ID NO: 69 - protein, 130 aa, synthetic construct
  REGION 1..130: note = synthetic construct; antigen binding domain
EVQLVESGGGLVQPGGSLRLSCAASGFTFSSYEMNWVRQAPGKGLEWVSYISSSGNTKDYAGSVKGRVTISRDNAKNLLYLQMNSLRAEDTAVYHCARDGGHYDILTGSMSYYYYALDVWGQGTTVTVSS

SEQ ID NO: 70 - protein, 108 aa, synthetic construct; identical to SEQ ID NO: 12
  REGION 1..108: note = synthetic construct; antigen binding domain

SEQ ID NO: 71 - protein, 121 aa, synthetic construct
  REGION 1..121: note = synthetic construct; antigen binding domain
EVQLVESGGGLVQPGGSLRLSCAASGFTFKTYAMSWVRQAPGRGLEWVSGISGSGSTSYYADSVKGRFTISRDNYKKTLSLQMNSLRAEDTAVYYCALDIMATVGGLFNNWGQGTLVTVSS

SEQ ID NO: 72 - protein, 108 aa, synthetic construct; identical to SEQ ID NO: 24
  REGION 1..108: note = synthetic construct; antigen binding domain

SEQ ID NO: 73 - protein, 120 aa, synthetic construct
  REGION 1..120: note = synthetic construct; antigen binding domain
QVQLVQSGAEVKKPGSSVKVSCKASGGTFSRHTISWVRQAPGQGLEWMGGIIPIFGTANYAHKFQGRVTITTDESTSTAYMELSSLRSEDTAVYYCARAPYTRQGYFDLWGRGTLVTVSS

SEQ ID NO: 74 - protein, 113 aa, synthetic construct
  REGION 1..113: note = synthetic construct; antigen binding domain
DIVMTQSPDSLAVSLGERATINCKSSQSVLYSSNNKNYLAWYQQKPGQPPKLLIYWASTRESGVPDRFSGSGSGTDFTLTISSLQAEDVAVYYCQQDYSTPWTFGQGTKVEIK

SEQ ID NO: 75 - protein, 118 aa, synthetic construct
  REGION 1..118: note = synthetic construct; antigen binding domain
QVQLVQSGAEVKKPGASVKVSCKASGYTFTNYYIHWVRQAPGQGLDWMGIINPGGGNTNYAQKFLGRVTMTRDTSTTTVYMELSSLRSEDTAIYYCARENWNSYFDNWGQGTLVTVSS

SEQ ID NO: 76 - protein, 113 aa, synthetic construct
  REGION 1..113: note = synthetic construct; antigen binding domain
DIVMTQSPDSLAVSLGERATINCKSSQSVLYSSNNKNFLAWYQQKPGQPPKLLIYWASTRESGVPDRFSGSGSGTDFTLTISSLQAEDVALYYCQQYYGAPWTFGQGTKVEIK

SEQ ID NO: 77 - protein, 119 aa, synthetic construct
  REGION 1..119: note = synthetic construct; antigen binding domain
QVQLVQSGAEVKKPGSSVKVSCKASGGTFSSYTINWVRQAPGQGLEWMGGIIPIFGIANYAQKFQGRVTITTDESTNTAYMELSSLRSEDTAIYYCARARYGSGSYDYWGQGTLVTVSS

SEQ ID NO: 78 - protein, 113 aa, synthetic construct
  REGION 1..113: note = synthetic construct; antigen binding domain
DIVMTQSPDSLAVSLGERATINCKSSQSVLYTSNNKNYLAWYQQKPGQPPKLLIYWASTRESGVPDRFSGSGSGTDFTLTISSLQAEDVAVYYCQQYYNTPWTFGQGTKVEIK

SEQ ID NO: 79 - protein, 120 aa, synthetic construct
  REGION 1..120: note = synthetic construct; antigen binding domain
QITLKESGPTLVKPTQTLTLTCTFSGFSLSTNGVGVGWIRQPPGKALEWLGIIYWNDDKRYSPSLRSRLTITKDTSKNQVVLTMTNMDPVDTATYYCAHRGLFGGWFDPWGQGTLVTVSS

SEQ ID NO: 80 - protein, 107 aa, synthetic construct
  REGION 1..107: note = synthetic construct; antigen binding domain
DIQMTQSPSSLSASVGDRVTITCRASQSISRYLNWYQQKPGKAPNLLIFAASSLQSGVPSRFSGSGSGTDFTLTISSLQPEDFATYFCQQSYNTPLTFGGGTKVEIK

SEQ ID NO: 81 - protein, 122 aa, synthetic construct
  REGION 1..122: note = synthetic construct; antigen binding domain
EVQLVESGGGLVQPGGSLRLSCAISGFTFRSYAMTWVRQAPGKALEWVSVISGSGGNTYYADSVKGRFTVSRDNSRNTLYLQMNSLRAEDTAVYFCSKVAAANNYYYALDVWGQGTTVTVSS

SEQ ID NO: 82 - protein, 112 aa, synthetic construct
  REGION 1..112: note = synthetic construct; antigen binding domain
DIVMTQSPLSLPVTPGEPASISCRSSQSLLHSNGYKYLDWYLQKPGQSPQLLIYLVSNRASGVPDRFSGSGSGTDFTLKISRVEAEDVGVYYCMQALQTPYTFGQGTKLEIK

SEQ ID NO: 83 - protein, 127 aa, synthetic construct
  REGION 1..127: note = synthetic construct; antigen binding domain
QVQLVESGGGVVQPGRSLRLSCVASGFTFSNYGMHWVRQAPGKGLEWVAVIWNDGSNKYYADSVKGRFTISRDNSKNTLYLQVSSLRADDTAVYYCARDGEVEYSSSNYNYYGLDVWGQGTTVTVSS

SEQ ID NO: 84 - protein, 107 aa, synthetic construct
  REGION 1..107: note = synthetic construct; antigen binding domain
DIQMTQSPSSLSASVGDRVTITCQASQDISNYLNWYQQKPGKAPKLLIYDASNLETGVPSRFSGSGSGTDFTFTISSLQPEDIVTYYCQQYDDLPITFGQGTRLEIK

SEQ ID NO: 85 - protein, 125 aa, synthetic construct
  REGION 1..125: note = synthetic construct; antigen binding domain
EVQLVESGGGLVQPGGSLRLSCAASGFSFHNFAMNWVRQAPGKGLEWVSVITGSGTSTHYADSVKGRFTISRDNSKKTLYLQMNSLRAEDTAVYYCAKDRGYDYSGSYYNWFDPWGQGTLVTVSS

SEQ ID NO: 86 - protein, 109 aa, synthetic construct
  REGION 1..109: note = synthetic construct; antigen binding domain
DIQMTQSPSSLSASVGDRITITCRASQSISSYLNWYQQKPGKAPKLLIFAASNLQSGVPSRFSGSGSGTDFTLTISSLQPEDFATYYCQQSYSTPSLFTFGPGTKVDIK

SEQ ID NO: 87 - protein, 128 aa, synthetic construct
  REGION 1..128: note = synthetic construct; antigen binding domain
EVQLVESGGGLVQPGGSLRLSCAVSGFTFSSYEMNWVRQAPGKGLEWVSHISSSGSTIYYADSVKGRFTMSRDNAKNSLYLQMNSLRAEDTAVYYCARDGNIWSGYYAAYYFYGMDVWGQGTTVTVSS

SEQ ID NO: 88 - protein, 112 aa, synthetic construct
  REGION 1..112: note = synthetic construct; antigen binding domain
DIVMTQTPLSSPVTLGQPASISCRSSQSLVHSDGKTYLSWLQQRPGQPPRLLIYKISNRFSGVPDRISGSGAGTDFTLKISRVEAEDVGVYYCMQAVQFPRTFGQGTKVEIK

SEQ ID NO: 89 - protein, 122 aa, synthetic construct
  REGION 1..122: note = synthetic construct; antigen binding domain
QVQLQQWGAGLLNPSETLSLTCAVYGGAFSDYYWNWIRQPPGKGLEWIGEINHRGSTNYNPSLKSRVTISVDTSKNQFSLRMSSVTAADAAVYYCARGEDYDIWNGYYQEKWGQGTLVTVSS

SEQ ID NO: 90 - protein, 107 aa, synthetic construct
  REGION 1..107: note = synthetic construct; antigen binding domain
EIVLTQSPATLSLSPGERATLSCRASQSISTYLAWYQQKPGQAPRLLIYDASKRATGIPARFSGSGSGTDFTLTISSLEPEDFVVYYCHQRSNWPLTFGGGTKVEIK

SEQ ID NO: 91 - protein, 117 aa, synthetic construct
  REGION 1..117: note = synthetic construct; antigen binding domain
QVQLQESGPGLVKPSETLSLTCTVSGGSFSSYYWSWLRQPPGKGLEWIGYIFYSGSTDYNPSLKSRVTISVDTSKKQFSLKLTSVTAADTAVYYCARTISTWWFAPWGQGTLVTVSS

SEQ ID NO: 92 - protein, 106 aa, synthetic construct
  REGION 1..106: note = synthetic construct; antigen binding domain
EIVMTQSPATLSVSPGGRATLSCRASQSVSNNVAWYQQKPGQAPRLLIYGASTRATGIPGRFSGSGSGTEFTLTISSLQSEDFAVYSCQQYNNWLTFGGGTKVEIK

SEQ ID NO: 93 - protein, 123 aa, synthetic construct
  REGION 1..123: note = synthetic construct; antigen binding domain
QVQLVESGGGVVQPGRSLRLSCVASGFTFSSYGMHWVRQAPGKGLEWVAIIWYDGSNKYYADSVKGRFTISRDNSKNTQYLQMNSLRAEDTAVYYCASVATSGDFDYYGMDVWGQGTTVTVSS

SEQ ID NO: 94 - protein, 107 aa, synthetic construct
  REGION 1..107: note = synthetic construct; antigen binding domain
EIVLTQSPATLSLSPGERTTLSCRASQRISTYLAWYQQKPGQAPRLLIYDASKRATGIPARFSGSGSGTGFTLTISSLEPEDFAVYYCQQRSNWPLTFGGGTKVEIK

SEQ ID NO: 95 - protein, 119 aa, synthetic construct
  REGION 1..119: note = synthetic construct; antigen binding domain
EVQLVQSGAEVRKPGESLKISCKGSGYSFTNYWIVWVRQMPGKGLEWMGIIYPGDSDTRYSPSFQGQVTISADKSISTAYLQWSSLKASDTAMYYCARRDTIFPSYPLWGQGTLVTVSS

SEQ ID NO: 96 - protein, 112 aa, synthetic construct
  REGION 1..112: note = synthetic construct; antigen binding domain
DIVMTQSPLSLPVTPGEPASISCRSSQSLLNSNGYNFLDWYLQKPGQSPQLLIYLVSNRASGVPDRFSGSGSGTDFTLKISRVEAEDIGVYYCMQALQTPITFGQGTRLEIK

SEQ ID NO: 97 - protein, 120 aa, synthetic construct
  REGION 1..120: note = synthetic construct; antigen binding domain
QITLKESGPTLVKPTQTLTLTCTFSGFSLSTNGVGVGWIRQPPGKALEWLTLIYWNENKHYSPSLKNRITITKDTSKNQVVLTMTNLDPVDTATYYCVHRGWLGAIFAYWGQGTLVTVSS

SEQ ID NO: 98 - protein, 108 aa, synthetic construct; identical to SEQ ID NO: 12
  REGION 1..108: note = synthetic construct; antigen binding domain

SEQ ID NO: 99 - protein, 126 aa, synthetic construct
  REGION 1..126: note = synthetic construct; antigen binding domain
EVQLVESGGGLVQPGGSLRLSCAASGFTFTSYAMTWVRQAPGKGLEWVSDISGSGGRTYYADSVKGRFTISRDNSKNMLYLQMNILRAEDTAVYHCAKGTGQQVDLYNYYYALDVWGQGTTVTVSS

SEQ ID NO: 100 - protein, 129 aa, synthetic construct
  REGION 1..129: note = synthetic construct; antigen binding domain
QVQLVESGGGVVQPGRSLRLSCAASGFTFSYYGMHWVRQAPGKGLEWVAVIWYDGSNKHYADSVKGRFTISRDNSKNTLYLQMNSLRADDTAVYYCARDKGISGIKGGSYYYYYAMDVWGQGTTVTVSS

SEQ ID NO: 101 - protein, 120 aa, synthetic construct
  REGION 1..120: note = synthetic construct; antigen binding domain
EVQLVESGGGLVKPGGSLRLSCAASGFTFSNAWMTWVRQAPGKGLEWVGRIKNKIDGGTTDYAAPVKGRFTISRDDSKNTVYLQMNSLKTEDTAVYYCSTVDYNWYFDFWGRGTLVTVSS

SEQ ID NO: 102 - protein, 129 aa, synthetic construct
  REGION 1..129: note = synthetic construct; antigen binding domain
QVQLVESGGGVVQPGRSLRLSCAASGFTFSFFGMHWVRQAPGKGLEWVALIWYDGTNENYADSVKGRFTISRDNSKSTLYLQMNSLRAEDTAVYYCARDRGVATFTRGNYYYNYGMDVWGQGTTVTVSS

SEQ ID NO: 103 - protein, 129 aa, synthetic construct
  REGION 1..129: note = synthetic construct; antigen binding domain
QVQLVESGGGVVQPGRSLRLSCAASGFTFSFYGMHWVRQAPGKGLEGVAVIWYDGSNKYYADSVKGRFTISRDNSKNMLYLQMTSLRAEDTAVYYCARDSGKTGTGITGYSYYYGMDVWGQGTTVTVSS

SEQ ID NO: 104 - protein, 118 aa, synthetic construct
  REGION 1..118: note = synthetic construct; antigen binding domain
QLQLQESGPGLVKPSETLSLTCTVSGGSIITNSYYWGWIRQPPGKGLEWIGSIYYSGRTYYNPSLESRVTISVDTSKNQFSLKLTSVTAADTAIYYCAREGDPSLDPWGQGTLVTVSS

SEQ ID NO: 105 - protein, 108 aa, synthetic construct; identical to SEQ ID NO: 24
  REGION 1..108: note = synthetic construct; antigen binding domain

SEQ ID NO: 106 - protein, 121 aa, synthetic construct
  REGION 1..121: note = synthetic construct; antigen binding domain
EVQLVESGGDLVQPGGSLRLSCAASGFTFSTYAMNWVRQAPGKGLEWVSHISGSGGNSYSADSVKGRFTISRDNSKNTLYLQMNSLRAEDTAIYYCSLDIMATVGGLFAYWGQGTLVTVSS

SEQ ID NO: 107 - protein, 131 aa, synthetic construct
  REGION 1..131: note = synthetic construct; antigen binding domain
QVQLVESGGGVVQPGRSLRLSCVASGFIFSFYGMHWVRQAPDKGLEWVAVIWYDGSNEYYADSVKGRFTISRDNSKNTLYLQMNSLRAEDTAVYYCGRDQGISYYDILTGNYNYYYGVDVWGQGTTVTVSS

SEQ ID NO: 108 - protein, 119 aa, synthetic construct
  REGION 1..119: note = synthetic construct; antigen binding domain
QVQLQQWGAGLLKPSETLSLTCAVYGGSFSGYYWNWIRQPPGKGLEWVGEISHRGSTNYNPSLKSRVTISLDTSKNQFSLKLTSVTAADTAVYYCSRDEELEFRFFDYWGQGTLVTVSS

SEQ ID NO: 109 - protein, 107 aa, synthetic construct; identical to SEQ ID NO: 46
  REGION 1..107: note = synthetic construct; antigen binding domain

SEQ ID NO: 110 - protein, 124 aa, synthetic construct
  REGION 1..124: note = synthetic construct; antigen binding domain
EVQLVESGGGLVQPGGSLRLSCVASGFTFSLYAMTWVRQVPGKGLEWVSTISGSGGGTYYTDSVKGRFTISRDNSKNTLYLQMNSLRADDTAVFYCTKESTTGTYSYFYGMDVWGQGTTVTVSS

SEQ ID NO: 111 - protein, 107 aa, synthetic construct
  REGION 1..107: note = synthetic construct; antigen binding domain
DIQMTQSPSSLSASVGDRVTITCRASQTISSYLNWYQQKPGKAPKLLIYAASSLQSGVPSRFSGSGSGTDFTLTLSGLQPEDFATYYCQQSYSTPLTFGGGTKVEIK

SEQ ID NO: 112 - protein, 121 aa, synthetic construct
  REGION 1..121: note = synthetic construct; antigen binding domain
EVQLVESGGGLVQPGGSLRLSCAASGFTFSRFWMSWVRQAPGKGLEWVANINQDGTEKYYVDSVKGRFTISRDNAKNSLYLQMNSLRAGDTAVYYCANTYYDFWSGHFDYWGQGTLVTVSS

SEQ ID NO: 113 - protein, 107 aa, synthetic construct
  REGION 1..107: note = synthetic construct; antigen binding domain
DIQMTQSPSTLSASVGDRVTITCRASQSISNWLAWYQQKPGKAPKLLIYKASSLESGVPSRFSGSGSGTEFTLTISSLQPDDFATYYCQQYHSYSYTFGQGTKLEIK

SEQ ID NO: 114 - protein, 121 aa, synthetic construct
  REGION 1..121: note = synthetic construct; antigen binding domain
QEHLVESGGGVVQPGRSLRLSCEASGFTFSNFGMHWVRQAPGKGLEWVAALWSDGSNKYYADSVKGRVTISRDNSKNTLYLQMNSLRAEDTAVYYCARGRGAPGIPIFGYWGQGTLVTVSS

SEQ ID NO: 115 - protein, 107 aa, synthetic construct
  REGION 1..107: note = synthetic construct; antigen binding domain
DIQMTQSPSSLSASVGDRVTITCRASQGIRNDLGWYQQKPGKAPKRLIYTASSLQSGVPSRFSGSGSGTEFTLTISSLQPEDFATYYCLQHNSYPLTFGGGTKVAIK

SEQ ID NO: 116 - protein, 130 aa, synthetic construct
  REGION 1..130: note = synthetic construct; antigen binding domain
EVQLVESGGGLVKPGGSLRLSCAASGFTFSNAWMSWVRQAPGKGLEWVGRIKRKTDGGTTDYAAPVKGRFTISRDDSKNTLHLQMNSLKTEDTAVYYCTTDDIVVVPAVMREYYFGMDVWGQGTTVTVSS

SEQ ID NO: 117 - protein, 107 aa, synthetic construct
  REGION 1..107: note = synthetic construct; antigen binding domain
DIQMTQSPSSLSASVGDRVTITCRTSQGIRNDLGWYQQKPGKAPKRLIYAASSLQSGVPSRFSGSGSGTEFTLTISSLQPEDFATYYCLQHNNYPYTFGQGTKLEIK

SEQ ID NO: 118 - protein, 121 aa, synthetic construct
  REGION 1..121: note = synthetic construct; antigen binding domain
QVQLVQSGAEVKKPGASVQVSCKASGYSFTGYYIHWVRQAPGQGLEWMGWINPNSGTKKYAHKFQGRVTMTRDTSIDTAYMILSSLISDDTAVYYCARDEDWNFGSWFDSWGQGTLVTVSS

SEQ ID NO: 119 - protein, 112 aa, synthetic construct
  REGION 1..112: note = synthetic construct; antigen binding domain
DIVMTQTPLSSPVTLGQPASISCRSSQTLVHGDGNTYLSWIQQRPGQPPRLLIYKVSNQFSGVPDRFSGSGAGTDFTLKISRVEAEDVGLYFCMQATHFPITFGQGTRLEIK

SEQ ID NO: 120 - protein, 121 aa, synthetic construct
  REGION 1..121: note = synthetic construct; antigen binding domain
QVHLVQSGAEVKKPGASVKVSCKASGYTFTGYYIHWVRQAPGHGLEWMGWLNPNTGTTKYIQNFQGRVTMTRDTSSSTAYMELTRLRSDDTAVYYCARDEDWNYGSWFDTWGQGTLVTVSS

SEQ ID NO: 121 - protein, 112 aa, synthetic construct
  REGION 1..112: note = synthetic construct; antigen binding domain
DIVMTQTPLSSPVTLGQPASISCRSSPSLVHSDGNTYLSWLQQRPGQPPRLLIYKISNRFSGVPDRFSGSGAGTDFTLKISRVEAEDVGVYYCMQATHFPITFGQGTRLEIR

SEQ ID NO: 122 - protein, 120 aa, synthetic construct
  REGION 1..120: note = synthetic construct; antigen binding domain
EVQLVESGGGVVRPGGSLRLSCAASGFTFDDYGMTWVRQAPGRGLEWVSGIHWHGKRTGYADSVKGRFTISRDNAKKSLYLQMNSLKGEDTALYHCVRGGMSTGDWFDPWGQGTLVIVSS

SEQ ID NO: 123 - protein, 108 aa, synthetic construct
  REGION 1..108: note = synthetic construct; antigen binding domain
DIQMTQSPSSLSASLGDRVTITCRASQSINSYLNWYQQKPGKAPKLLIYVASSLQSGVPSRFSGSGSGTEFTLTISNLQPEDFATYYCQQSYSTPPITFGQGTRLEIK

SEQ ID NO: 124 - protein, 120 aa, synthetic construct
  REGION 1..120: note = synthetic construct; antigen binding domain
EVQLVESGGGVVRPGGSLRLSCAASGFTFDDYGMTWVRQVPGKGLEWVSGIHWSGRSTGYADSVKGRFTISRDNAKNSLYLQMNSLRAEDTALYYCARGGMSTGDWFDPWGQGTLVTVSS

SEQ ID NO: 125 - protein, 108 aa, synthetic construct
  REGION 1..108: note = synthetic construct; antigen binding domain
DIQMTQSPSSLSASVGDRVTITCRASQSISSYLNWYQQKPGKAPKLLIYVASSLQSGVPSRFSGSGSGTDFTLTISSLQPEDFATYYCQQSYSTPPITFGQGTRLEIK

SEQ ID NO: 126 - protein, 115 aa, synthetic construct
  REGION 1..115: note = synthetic construct; antigen binding domain
EVQLVESGGGLVQPGGSLRLSCAASGFTVGSNYMNWVRQAPGKGLEWVSVIYSGGSTYYADSVKGRFTISRLTSKNTLYLQMSSLRPEDTAVYYCARGIRGLDVWGQGTTVTVSS

SEQ ID NO: 127 - protein, 108 aa, synthetic construct
  REGION 1..108: note = synthetic construct; antigen binding domain
DIQMTQSPSSLSASVGDRVTITCRASQTINIYLNWYQQKPGRAPRLLIYAASSLQSGVPSRFSGSGSGTDFTLTISSLQPEDFATYYCHQSYSTPPITFGQGTRLEIK

SEQ ID NO: 128 - protein, 115 aa, synthetic construct
  REGION 1..115: note = synthetic construct; antigen binding domain
EERLVESGGDLVQPGGSLRLSCAASGITVGTNYMNWVRQAPGKGLEWVSVISSGGNTHYADSVKGRFIMSRQTSKNTLYLQMNSLETEDTAVYYCARGIRGLDVWGQGTMVTVSS

SEQ ID NO: 129 - protein, 108 aa, synthetic construct
  REGION 1..108: note = synthetic construct; antigen binding domain
DIQMTQSPSSLSASVGDRVTITCRASQSMSSYLNWYQQKPGRAPKLLIFAASSLQSGVPSRFSGSGSGTDFTLTISSLQPEDFATYYCQQSYSTPPITFGQGTRLEIK

SEQ ID NO: 130 - protein, 118 aa, synthetic construct
  REGION 1..118: note = synthetic construct; antigen binding domain
QVQLVQSGAEVKMPGSSVRVSCKASGGIFSSSTISWVRQAPGQGLEWMGEIIPVFGTVNYAQKFQDRVIFTADESTTTAYMELSSLKSGDTAVYFCARNWGLGSFYIWGQGTMVTVSS

SEQ ID NO: 131 - protein, 108 aa, synthetic construct
  REGION 1..108: note = synthetic construct; antigen binding domain
EIVLTQSPGTLSLSPGERATLSCRASQSFNFNYLAWYQQKPGQAPRLLIYGASSRATGIPDRFSGSGSGTDFTLTINRLEPEDFGVFYCQQYESAPWTFGQGTKVEIK

SEQ ID NO: 132 - protein, 115 aa, synthetic construct
  REGION 1..115: note = synthetic construct; antigen binding domain
EVQLVESGGDLVHPGRSLRLSCAASGFPFDEYAMHWVRQVPGKGLEWVSGISWSNNNIGYADSVKGRFTISRDNAKNSLYLQMNSLRPEDTAFYYCAKSGIFDSWGQGTLVTVSS

SEQ ID NO: 133 - protein, 105 aa, synthetic construct
  REGION 1..105: note = synthetic construct; antigen binding domain
DIQMTQSPSSLSASVGDRVTITCRASQSISSYLNWYQQKPGKLLIYAASSLQSGVPSRFSGGGSGTDFTLTISSLRPEDFATYYCQQSYCTPPITFGQGTRLEIK

SEQ ID NO: 134 - protein, 118 aa, synthetic construct
  REGION 1..118: note = synthetic construct; antigen binding domain
EVQLVESGGGVVQPGRSLRLSCAASGFTFSSYGMHWVRQAPGKGLEWVTLISYEGRNKYYADSVKGRFTISRDNSKNTLYLQMNSLRAEDTAVYYCAKDRTLYGMDVWGQGTTVTVSS

SEQ ID NO: 135 - protein, 121 aa, synthetic construct
  REGION 1..121: note = synthetic construct; antigen binding domain
QVTLRESGPALVKTTQTLTLTCTFSGFSLSTNRMCVTWIRQPPGKALEWLARIDWDGVKYYNTSLKTRLTISKDTSKNQVVLTMTNMDPVDTATFYCARSTSLTFYYFDYWGQGTLVTVSS

SEQ ID NO: 136 - protein, 108 aa, synthetic construct; identical to SEQ ID NO: 12
  REGION 1..108: note = synthetic construct; antigen binding domain

SEQ ID NO: 137 - protein, 115 aa, synthetic construct
  REGION 1..115: note = synthetic construct; antigen binding domain
EVQLVESGGGLVQPGGSLRLSCAASEFTVGTNHMNWVRQAPGKGLEWVSVIYSGGNTFYADSVKGRFTISRHTSKNTLYLQMNSLTAEDTAVYYCARGLGGMDVWGQGTTVTVSS

SEQ ID NO: 138 - protein, 107 aa, synthetic construct
  REGION 1..107: note = synthetic construct; antigen binding domain
DIQMTQSPSSLSASVGDRVTITCRASQVISNYLAWYQQKPGKVPRLLIYAASTLQSGVPSRFSGSGSGTDFTLTISSLQPEDVATYYCQKYNSAPRTFGQGTKVEIK

SEQ ID NO: 139 - protein, 120 aa, synthetic construct
  REGION 1..120: note = synthetic construct; antigen binding domain
EVQLVESGGGLVQRGESLRLYCAASGFTFSKYWMNWVRQAPGKGLEWVANIKGDGSEKYYVDSVKGRFTISRDNAKNSLYLQMNSLRAEDTAVYYCARDYWGSGYYFDFWGQGTLVTVSS

SEQ ID NO: 140 - protein, 107 aa, synthetic construct
  REGION 1..107: note = synthetic construct; antigen binding domain
DIQMTQSPSSLSASVGDRVTITCRASQNINNYLNWYQQKPGKAPKLLIYAASSFQNAVPSRFSGSGSGTDFTLTISSLQPEDFATYYCQQSYNTPLTFGGGTKVEIK

SEQ ID NO: 141 - protein, 130 aa, synthetic construct
  REGION 1..130: note = synthetic construct; antigen binding domain
EVQLVESGGGLVQSGGSLRLSCAASGFTFSSYWMSWVRQAPGKGLEWVANIKQDGSEKYYVDSVKGRFTISRDNAKNSLYLQMNSLRADDTAVYYCARDDIVVVPAPMGYYYYYFGMDVWGQGTTVTVSS

SEQ ID NO: 142 - protein, 107 aa, synthetic construct
  REGION 1..107: note = synthetic construct; antigen binding domain
DIQMTQSPSSLSASVGDRVTITCRASQGIRNDLGWYQQKPGKAPKRLIYAASSLQSGVPSRFSGSGSGTEFTLTISSLQPEDFATYYCLQHNSYPYTFGQGTKLEIK

SEQ ID NO: 143 - protein, 123 aa, synthetic construct
  REGION 1..123: note = synthetic construct; antigen binding domain
EVQLVESGGGLVQPGRSLRLSCAASGFTFDDFAMHWVRQAPGKGLEWVSGISWTGGNMDYANSVKGRFTISREDAKNSLYLQMNSLRAADTALYYCVKDIRGIVATGGAFDIWGRGTMVTVSS

SEQ ID NO: 144 - protein, 107 aa, synthetic construct
  REGION 1..107: note = synthetic construct; antigen binding domain
DIQMTQSPSSLSASVGDRVTISCRASQTISTYLNWFQQKPGKAPKLLIYVVSSLQSGVPSRFSGSGSGTDFTLTISSLQPEDFATYYCQQSYSTPFTFGPGTKVDIK

SEQ ID NO: 145 - protein, 115 aa, synthetic construct
  REGION 1..115: note = synthetic construct; antigen binding domain
EVQLVESGGGLVQPGGSLRLSCAASGFTVGTNYMNWVRQAPGKGLEWISVIYSGGSTFYADSVKGRFTISRQTSQNTLYLQMNSLRPEDTAVYYCARGIRGFDIWGQGTMVTVSS

SEQ ID NO: 146 - protein, 108 aa, synthetic construct; identical to SEQ ID NO: 12
  REGION 1..108: note = synthetic construct; antigen binding domain

SEQ ID NO: 147 - protein, 115 aa, synthetic construct
  REGION 1..115: note = synthetic construct; antigen binding domain
EVQLVESGGGLVQPGGSLRLSCAASGFTISTNYMNWVRQAPGKGLEWVAVIYSSGSTYYIDSVKGRFTISRLTSKNTVYLQMSSLNSEDTAVYYCARGIRGFDIWGQGTMVTVSS

SEQ ID NO: 148 - protein, 124 aa, synthetic construct
  REGION 1..124: note = synthetic construct; antigen binding domain
EVQLVESGGGLVQPGRSLRLSCAASGFTIDDSAMHWVRQTPGKGLEWVSGISWKSGSIGYADSVRGRFTISRDNAKNSLYLQMNSLRVEDTALYYCVKDIRGNWNYGGNWFDPWGQGTLVTVSS

SEQ ID NO: 149 - protein, 115 aa, synthetic construct
  REGION 1..115: note = synthetic construct; antigen binding domain
EVQLVESGGGLVQPGGSLRLSCEASGFTVGVNHMNWVRQAPGKGLEWVSVIFSSGRTFYGDYVKGRLTIFRQTSQNTVYLQMNSLRSEDTAIYYCARGIGGLDIWGRGTMVTVSS

SEQ ID NO: 150 - protein, 123 aa, synthetic construct
  REGION 1..123: note = synthetic construct; antigen binding domain
EVQLVESGGGLVQPGRSLRLSCAASGFTFDDYALHWVRQAPGKGLEWVSGISWTGGTIDYADSVKGRFTISRDNAKNSLYLQMSSLRTEDTAIYYCTRDIRGNWKYGGWFDPWGQGTLVTVSS

SEQ ID NO: 151 - protein, 120 aa, synthetic construct
  REGION 1..120: note = synthetic construct; antigen binding domain
QVQLVQSGTEVKKPGASVKVSCKASGYTFTAYYMHWVRQAPGQGLDWMGWISPNSGFTNYAQKFQGRVTMTRDTSINTFYMELSGLRSDDTAVYYCAREGSTHHNSFDPWGQGTLVTVSS

SEQ ID NO: 152 - protein, 114 aa, synthetic construct
  REGION 1..114: note = synthetic construct; antigen binding domain
EVQLVESGGGLVQPGGSLRLSCAASGFTVGTNFMNWVRQAPGKGLEWVSAIYSGGTANYADSVKGRFTISRDTSRNTLYLQMNSLRTEDTAVYYCARGGGMDVWGQGTTVTVSS

SEQ ID NO: 153 - protein, 118 aa, synthetic construct
  REGION 1..118: note = synthetic construct; antigen binding domain
QVQLVQSGAEVKKPGSSVKVSCKASGGTFNTYVLSWVRQAPGQGLEWMGEIIPILGAANYAQNFQGRVTFTTDESTNTAYMDLSSLRSEDTAVYYCARDRTSGGFDPWGQGTLVTVSS

SEQ ID NO: 154 - protein, 119 aa, synthetic construct
  REGION 1..119: note = synthetic construct; antigen binding domain
QVQLVQSGAEVEKPGASVKVSCKASGYIFTHYGISWVRQAPGQGLEWVGWISPYNGYTDYAQKLQGRVTLTTDTSTTTAYMELRNLRSDDTAMYYCSRGRGPYWSFDLWGRGTLVTVSS

SEQ ID NO: 155 - protein, 117 aa, synthetic construct
  REGION 1..117: note = synthetic construct; antigen binding domain
QVQLVQSGAEVKKPGASVKVSCKASDYTFTSYGISWVRQAPGQGLEWMGWISVYNGNINYAQKFKGRVTMTTDTSTSTAYMELRSLRSDDMAVYYCARVTQFGMDVWGQGTTVTVSS

SEQ ID NO: 156 - protein, 107 aa, synthetic construct
  REGION 1..107: note = synthetic construct; antigen binding domain
DIQMTQSPSSLSASVGDRVTITCRASQSISSNLNWYQQNPGKAPKLLIYTTSSLQGGVPSRFSGSGSGTDFTLTISSLQPEDFATYYCQQSFRTPFTFGPGTKVDIK

SEQ ID NO: 157 - protein, 128 aa, synthetic construct
  REGION 1..128: note = synthetic construct; antigen binding domain
EVQLVESGGGLVQPGGSLKLSCAASGFTFSGSAMHWVRQASGKGLEWVGRIRGKANSFATAYSASVKGRFTISRDDSKNTASLQMNSLRTEDTAVYFCTREDQQLVRPYYYHYGMDVWGQGTTVTVSS

SEQ ID NO: 158 - protein, 107 aa, synthetic construct
  REGION 1..107: note = synthetic construct; antigen binding domain
DIQMTQSPSSLSASVGDRVTITCRTSQSITNYLNWYQQKPGKAPKLLIYATASLQSGVPSRFSGSGSETDFTLTISSLQPEDFATYYCQQSYSTPLTFGGGTKVEIK

SEQ ID NO: 159 - protein, 123 aa, synthetic construct
  REGION 1..123: note = synthetic construct; antigen binding domain
QITLKESGPTLVKPTQTLTLTCTFSGFSLSTSGVGVGWIRQSPGRALEWLALIYWNDHERYSPSLKSRLTITKDTSKNLVVLAMANMDPVDTATYFCAHRNIEYRRSYFFDYWGQGTLVTVSS

SEQ ID NO: 160 - protein, 107 aa, synthetic construct
  REGION 1..107: note = synthetic construct; antigen binding domain
DIQMTQSPSSVSASVRDRVTVTCRASQDINNWLAWYQQKPGKAPKLLIYAASSLQSGVPSRFSGSGSGTDFTLTISSLQPEDFATYYCQQANTFPFTFGPGTKVDIK

SEQ ID NO: 161 - protein, 118 aa, synthetic construct
  REGION 1..118: note = synthetic construct; antigen binding domain
QVQLQESGPGLVKPSETLSLTCTVSGGSINSYYWTWIRQPPGKGLEWIGYVYYSGSTTYNPSLKSRVTISVDTSKNQFFLNLNSVTAAETAVYYCARGTLGYYGMDVWGQGTTVTVSS

SEQ ID NO: 162 - protein, 108 aa, synthetic construct
  REGION 1..108: note = synthetic construct; antigen binding domain
EIVLTQSPGTLSLSPGERATLSCRASQSFSNNYLAWYQQKPGQAPRLLIYGTSIRATGIPDRFSGSGSGTDFTLAISRLEPEDFAVYYCQQYGRSPLTFGGGTKVEIK

SEQ ID NO: 163 - protein, 118 aa, synthetic construct
  REGION 1..118: note = synthetic construct; antigen binding domain
QVQLVESGGGVVQPGRSLRLSCAASGFTFSSYGMNWVRQAPGKGLEWVAVTWYDGSNKHYADSVKGRFTISRDNSKNTLYLQMYSLRAEDTAMYYCVRGGHLGAFDIWGQGTMVTVSS

SEQ ID NO: 164 - protein, 107 aa, synthetic construct
  REGION 1..107: note = synthetic construct; antigen binding domain
EIVLTQSPGTLSLSPGERATLSCRASQSVSSYLAWYQQKPGQAPRLLIYGASSRATGIPDRFSGGGSGTDFTLTISRLEPEDFAVYYCQQYGSSPFTFGPGTKVDIK

SEQ ID NO: 165 - protein, 121 aa, synthetic construct
  REGION 1..121: note = synthetic construct; antigen binding domain
QVQLVQSGAEVKKPGASVKVSCKASGYTFTDYYIHWVRQAPGQGLEWMGWINPNNGVSNYAQKFQGRVTMTRDTSISTAYMDLIRLRSDDTAVYYCARERASWDYNGVDVWGQGTTVTVSS

SEQ ID NO: 166 - protein, 112 aa, synthetic construct
  REGION 1..112: note = synthetic construct; antigen binding domain
DIVMTQSPLSLPVTPGEPASISCRSSQSLLHSNGYSYLDWYLQKPGQSPQLLIYLGSNRASGVPDRFSGSGSGTDFTLKISRVEAEDVGVYYCMQGLQPPNTFGQGTKLEIK

SEQ ID NO: 167 - protein, 118 aa, synthetic construct
  REGION 1..118: note = synthetic construct; antigen binding domain
QLQLQESGPGLVKPSETLSLTCIVSGGSTSSNTYYWGWIRQPPGKGLEWIGTIHYSGNPYYDPSLKSRVTISVDTSKNHFSLKLNSVTAADTAVYYCTRQYINFFDFWGQGTLVTVSS

SEQ ID NO: 168 - protein, 107 aa, synthetic construct
  REGION 1..107: note = synthetic construct; antigen binding domain
EIVLTQSPATLSLSPGERVTLSCRASQSISRYLAWYQQKPGQAPRVLIYDASNRATDIPARFSGSGSGTDFTLTISSLEPEDFAVYYCQQRSNWPITFGQGTRLEIK

SEQ ID NO: 169 - protein, 121 aa, synthetic construct
  REGION 1..121: note = synthetic construct; antigen binding domain
QVQLVESGGGVVQPGRSLRLSCAASGLTFSYYGMHWVRQAPGKGLEWVAVISYDGSNKYYADSVKGRFTISRDNSKNTLYLQMNSLRAEDAAVYYCAKDLGGDDYYGMDVWGQGTTVTVSS

SEQ ID NO: 170 - protein, 108 aa, synthetic construct
  REGION 1..108: note = synthetic construct; antigen binding domain
EIVLTQSPGTLSLSPGERATLSCRASQSVSRTYLAWYQQKPGQAPRLLIYGAFSRATGIPDRFSGSGSGTDFTLTISRLEPEDFAVYYCQQYGSSPYTFGQGTKLEIK

SEQ ID NO: 171 - protein, 122 aa, synthetic construct
  REGION 1..122: note = synthetic construct; antigen binding domain
QVQLVESGGGLVKPGGSLRLSCAASGFTFSDYYMTWIRQAPGKGLEWVSYISSSGGNIFYADSVKGRFTISRDNAKNSLYLQMNSLRGEDTAVYYCARGLEPYHYYYGMDVWGQGTTVTVSS

SEQ ID NO: 172 - protein, 107 aa, synthetic construct
  REGION 1..107: note = synthetic construct; antigen binding domain
DIQMTQSPSSLSASVGDRVTITCQASQDISNYLNWYQQKPGKAPKLLIYDASNLETGVPSRFSGSGSGTDFTFTISSLQPEDIATYFCQHYDNLPFTFGPGTKVDIK

SEQ ID NO: 173 - protein, 123 aa, synthetic construct
  REGION 1..123: note = synthetic construct; antigen binding domain
EVQLVESGGGLVQPGGSLRLSCAASGFTLSNYVMTWVRQAPGKGLEWVSAISGRGGNSYYADSVKGRFSISRDHSKNTLYLQVNSLRAEDTAVYYCAKAERGYSYGFNWFDPWGQGTLVTVSS

SEQ ID NO: 174 - protein, 107 aa, synthetic construct
  REGION 1..107: note = synthetic construct; antigen binding domain
DIQMTQSPSSVSASAGDRVTITCRASQGISSWLAWYQQKPGKAPKLLIYAASSLQSGVPSRFSGSGSGTDFTLTISSLQPEDFASYYCQQGNNFPLTFGGGTKVEIK

SEQ ID NO: 175 - protein, 120 aa, synthetic construct
  REGION 1..120: note = synthetic construct; antigen binding domain
QVQLVESGGGVVQPGRSLRLSCAASGFTFSTYGMHWVRQAPGKGLEWVTVIWYDGNNKYYADSVKGRFTISRDNSKNTLYLQMNNLRAEDTALYYCARGGGRLSYYHDYWGQGTLVTVSS

SEQ ID NO: 176 - protein, 107 aa, synthetic construct
  REGION 1..107: note = synthetic construct; antigen binding domain
DIQMTQSPSSLSASVGDRVTITCRASQSISTFLNWYQQKPGKAPNLLIYGTSSLQSGVPSRFSGSGSGTDFTLTISSLQPEDFAAYYCQQTYSTPFTFGPGTKVDIK

SEQ ID NO: 177 - protein, 119 aa, synthetic construct
  REGION 1..119: note = synthetic construct; antigen binding domain
QVQLVQSGAEVKMSGASVRVSCKASGYTFTSYGISWMRQAPGQGLEWMGWITAYNGNSNYAQKLQGRVTMTTDTSTGTAYMELRSLTSDDTAVYYCARRGDYLGVFPYWGQGTLVTVSS

SEQ ID NO: 178 - protein, 107 aa, synthetic construct
  REGION 1..107: note = synthetic construct; antigen binding domain
DIQMTQSPSSLSASVGDRVTITCRASQSISSYLNWYQQKPGKAPNLLIYTASSLQSGVPSRFSGSGSGTDFTLTISSLQPEDFATYYCQQSYSSPLTFGGGTKVEIK

SEQ ID NO: 179 - protein, 116 aa, synthetic construct
  REGION 1..116: note = synthetic construct; antigen binding domain
EVQLVESGGGLVQPGGSLRLSCAASGFTFSNYEMSWVRQAPGKGLEWVSSIRTSGTTKYYADSMKGRFTISRDNAKNSLYLQMNSLRAEDTAVYYCAGGGTFLHYWGQGTLVTVSS

SEQ ID NO: 180 - protein, 108 aa, synthetic construct
  REGION 1..108: note = synthetic construct; antigen binding domain
DIQMTQSPSSVSASVGDRVTITCRASQGIASYLAWYQQKPGKAPKLLIYAASSLQTGVPSRFSGSGYGTDFTLTISSLQPEDFATYYCQQAKSFPMYTFGQGTKLEIK

SEQ ID NO: 181 - protein, 122 aa, synthetic construct
  REGION 1..122: note = synthetic construct; antigen binding domain
QVQLQESGPGLVKPSQTLSLTCTVSGGSITSGGYYWSWIRQHPGKGLEWIGYIFYSGITNYNPSLKSRVTISVDTSKNQFSLKLTSVTAADTAVYYCATYNSLRLYYGMDVWGQGTTVTVSS

SEQ ID NO: 182 - protein, 112 aa, synthetic construct
  REGION 1..112: note = synthetic construct; antigen binding domain
DVVMTQSPLSLPVILGQPASISCRSSQSLVYGDGNTYLNWFQQRPGQSPRRLIYKVSNRDSGVPDRFSGSGSGTDFTLKISRVEAEDVGVYYCMQSTHWPLTFGGGTKVEIK

SEQ ID NO: 183 - protein, 120 aa, synthetic construct
  REGION 1..120: note = synthetic construct; antigen binding domain
EVQLVESGGGLVQPGGSLRLACAASGFTFSDYYMDWVRQVPGKGLEWVGRSRDKANSFTTEYVASVKGRFTISREDSKNSVYLQMNSLKTEDTAVYYCARTNYDFSLDVWGQGTTVTVSS

SEQ ID NO: 184 - protein, 107 aa, synthetic construct
  REGION 1..107: note = synthetic construct; antigen binding domain
DIQMTQSPSSLSASVGDRVTITCRASQDINNYLAWFQQKPGNAPKSLIYAASSLQSGVPSKFSGSGSGTDFTLTISSLQPEDFATYYCQQYSTYPITFGQGTRLEIK

SEQ ID NO: 185 - protein, 118 aa, synthetic construct
  REGION 1..118: note = synthetic construct; antigen binding domain
QVQLQESGPGLVKPSETLSLTCTVSGGSISSYHWSWIRQPLGKGLEWIGYIYYSGSTNYNPSLKSRVTISVDTSKNQFSLKLSSVTAADTAVYYCARGGSSIWPFDYWGQGTLVTVSS

SEQ ID NO: 186 - protein, 107 aa, synthetic construct
  REGION 1..107: note = synthetic construct; antigen binding domain
DIQMTQSPSTLSASVGDRVTITCRASQSISSWLAWYQQKSGKAPKLLISKASTLESGVPSRFSGSGSGTEFTLTISSLQPDDFATYYCQQYNIYSWTFGQGTKVEIK

SEQ ID NO: 187 - protein, 120 aa, synthetic construct
  REGION 1..120: note = synthetic construct; antigen binding domain
QITLKESGPTLVKPTQTLTLTCTFSGFSLSTSGVGVGWIRQPPGVALEWLALIYWNDDKRFSPSLKSRLTITKDTSKNQVVLTMTNMDPVDTATYYCAHRRLGLYYFDYWGQGTLVTVSS

SEQ ID NO: 188 - protein, 107 aa, synthetic construct
  REGION 1..107: note = synthetic construct; antigen binding domain
DIQLTQSPSFLSASVGDRVTITCWASQGISSYLAWYQQKPGKAPKLLIYAASTLQSGVPSRFSGSGSGTEFTLTISSLQPEDFATYYCQQVHIYPFTFGPGTKVDIK

SEQ ID NO: 189 - protein, 122 aa, synthetic construct
  REGION 1..122: note = synthetic construct; antigen binding domain
QVQLVQSGAEVKKPGASVKVSCKASGYTLSSYGISWVRQAPGQGLEWMGWISAYNGNTNYAQKLQGRLTMTTDTSTSTAYMELRSLRSDDTAVYYCSRDGPFKISFFGMDVWGQGTTVTVSS

SEQ ID NO: 190 - protein, 108 aa, synthetic construct; identical to SEQ ID NO: 12
  REGION 1..108: note = synthetic construct; antigen binding domain

SEQ ID NO: 191 - protein, 118 aa, synthetic construct
  REGION 1..118: note = synthetic construct; antigen binding domain
QVQLVESGGGEVQPGRSLRLSCAASGFTFSSYGMHWVRQAPGKGLEWVAVIWYDGRNKHYVDSVKGRFTISRDNSKNTVYLQMNSLRAEDSAVYYCVRGGQLGAFDYWGQGTLVTVSS

SEQ ID NO: 192 - protein, 108 aa, synthetic construct; identical to SEQ ID NO: 24
  REGION 1..108: note = synthetic construct; antigen binding domain

SEQ ID NO: 193 - protein, 118 aa, synthetic construct
  REGION 1..118: note = synthetic construct; antigen binding domain
QVQLVESGGGVVQPGRSLRLSCAASGFTSSSYGIHWVRQAPGKGLEWVAVIWYDGSNKYYADSVKGRFTISRDNSKNTLYLQMNSLRAEDTAVYYCARGGPWGAFDIWGQGTMVTVSS

SEQ ID NO: 194 - protein, 108 aa, synthetic construct
  REGION 1..108: note = synthetic construct; antigen binding domain
DIRMTQSPSSLSASVGDRVTITCRASQTVNTFLNWYQQKPGKAPKLLIFGASSLQSGVPSRFSGSGSGTDFTLTISGLQPEDFAIYYCQQSYSVPPITFGQGTRLEIE

SEQ ID NO: 195 - protein, 122 aa, synthetic construct
  REGION 1..122: note = synthetic construct; antigen binding domain
QVQLHESGPGLVKPSQTLSLTCSVSGGSISNGGYYWSWIRQHPGQGLEWIGYIYYIGNTYYNPSLESRVTMSIDTSKNQFSLKLSSVTAADTAIYYCARQEFVPGAEYFLHWGQGILVTVSS

SEQ ID NO: 196 - protein, 107 aa, synthetic construct
  REGION 1..107: note = synthetic construct; antigen binding domain
DIQMTQSPSSLSASVGDRVTITCRASQDIRNDLGWHQQKSGKAPKSLIYAASSLQSGAPSRFSGSGSGTEFTLTISSLQPEDSATYYCLQQNSYPPTFGQGTKVEIK

SEQ ID NO: 197 - protein, 122 aa, synthetic construct
  REGION 1..122: note = synthetic construct; antigen binding domain
EVQLVESGGGLVQPGRSLRLSCAGTGFIFDDYAMHWVRQAPGKGLEWVSGISWNSNSLGYADSVKGRFTISRDNAKKSLYLQMSSLRAEDTALYYCVKDVTRLELRGFLDYWGQGTQVTVSS

SEQ ID NO: 198 - protein, 108 aa, synthetic construct
  REGION 1..108: note = synthetic construct; antigen binding domain
EIVLTQSPDTLSLSPGERATLSCRASQSVSSSFLAWYQQKPGQAPRLLIYGASSRATGIPDRFSGSGSGTDFTLTISRLEPEDFAVYYCQQYGRSPWTFGQGTKVAIK

SEQ ID NO: 199 - protein, 118 aa, synthetic construct
  REGION 1..118: note = synthetic construct; antigen binding domain
DRQMVESGGGVVQPGRSLRLSCIASGFIISRYGMHWVRQAPGKGLEWVAVIWYDGRNKNYADSVKGRFTISRDNSKNTLYLEMNSLRAEDTAVYYCGRVHQFGAFDIWGQGTMVTVSS

SEQ ID NO: 200 - protein, 108 aa, synthetic construct
  REGION 1..108: note = synthetic construct; antigen binding domain
DIQMTQSPSSLSASVGDRITITCRGSQNIGSFLSWYQQRPGKAPKLLIFGAYNLQGGVPSRFSGSGSGTDFTLTISSLQPEDFATYFCQQSYSTPPITFGQGTRLEIK

SEQ ID NO: 201 - protein, 121 aa, synthetic construct
  REGION 1..121: note = synthetic construct; antigen binding domain
QVQLQESGPGLVKPSQTLSLTCTVSGGSINNGGHYWTWIRQHPGKGLEWIGYIYYIGTTYYNPSLESRLSLSVDTSKNQFSLKLSSVTAADTAIYYCARSSLSVSEAFDVWGQGTMVTVSS

SEQ ID NO: 202 - protein, 108 aa, synthetic construct
  REGION 1..108: note = synthetic construct; antigen binding domain
DIQMTQSPSSLSASVGDRFTITCRASQSIGSFLSWYQQKPGKAPKLLIYAASSLQSGVPSRFSGSGSGTDFTLTISSLQPEDFATYYCQQSYNTPPITFGQGTRLEIK

SEQ ID NO: 203 - protein, 121 aa, synthetic construct
  REGION 1..121: note = synthetic construct; antigen binding domain
QVQLQESGPGLVRPSQTLSLTCTVSGGSISNGGYYWTWIRQNPGKGLEWIGYIYYIGTTYYNPSLESRLSLSVDTSKNQFSLKLTSVTAADTAVYYCARSSLAVSEAFDIWGQGTMVTVSS

SEQ ID NO: 204 - protein, 108 aa, synthetic construct
  REGION 1..108: note = synthetic construct; antigen binding domain
DIQLTQSPSSLSASVGDRVTITCRASQTISTYLNWYQQKPGNAPKLLIYAASSLQSGVPSRFSGRGSGTDFTLTISSLQPEDFATYYCQQGYTTPPITFGQGTRLEIK

SEQ ID NO: 205 - protein, 121 aa, synthetic construct
  REGION 1..121: note = synthetic construct; antigen binding domain
QVQLVQSGTEVKRPGASVKVSCKASGFTFTGYYIYWVRQAPGEGLEWMGWINPHSGGTKYAQKFQGRVTLTRDTSINTAYLDLISLRSDDTAVYYCARIGGGGYSSYFDYWGQGTLVTVSS

SEQ ID NO: 206 - protein, 107 aa, synthetic construct
  REGION 1..107: note = synthetic construct; antigen binding domain
DIQMTQSPSSVSASVGDRVTITCRASQDISSWLAWYQQKPGKAPKLLIYTTANLQSGVPSRFSGSGSGTDFTLTISSLQSEDFATYYCQQANSFPFTFGSGTKVDIK

SEQ ID NO: 207 - protein, 121 aa, synthetic construct
  REGION 1..121: note = synthetic construct; antigen binding domain
EVQLLESGGGLVQPGGSLRLSCAASGFTFSSYAMSWVRQAPGKGLEWVSDISGSGLSTYYADSVKGRFAISRDNSKNMLYLQMNRLRAEDTAVYYCAKEPSHWNGEAFDIWGQGTMVTVSS

SEQ ID NO: 208 - protein, 108 aa, synthetic construct
  REGION 1..108: note = synthetic construct; antigen binding domain
EIVLTQSPDTLSLSPGERATLSCRASQTVSNSHLAWYQQKPGQAPRLLIYGTSSRATGIPDRFSGSGSGTDFSLTIIRLEPDDFAVYFCQQHESSPPTFGQGAKLEIK

SEQ ID NO: 209 - protein, 122 aa, synthetic construct
  REGION 1..122: note = synthetic construct; antigen binding domain
QLQLQESGPGLVKPSETLSFTCTVSGGSISSNYYYWGWVRQSPGKGLEWIGSIYHTGNAYDNPSLKSRVTISVDTSKNQFSLNLNSVTAADTAIYYCARHHSSSSWWYFDVWGRGTLVIVSS

SEQ ID NO: 210 - protein, 108 aa, synthetic construct
  REGION 1..108: note = synthetic construct; antigen binding domain
EIVLTQSPGTLSLSPGERATLSCRASQWISSSYLAWYQQKPGQAPRLLIYGAFSRAPGIPGRFSGSGSGTDFTLTISRLEPEDFAVYYCQQYGSSPYTFGQGTKLEIN

SEQ ID NO: 211 - protein, 121 aa, synthetic construct
  REGION 1..121: note = synthetic construct; antigen binding domain
QVQLVESGGGVVQPGRSLRLSCAASGITFSSYGMHWVRQAPGKGLEWVALTSYDGSKKYYSDSVKGRFTISRDNSKNTLYLQMNSLRPEDTAVYYCAKDKGGDDYYGMDVWGQGTTVTVSS

SEQ ID NO: 212 - protein, 108 aa, synthetic construct
  REGION 1..108: note = synthetic construct; antigen binding domain
DIQMTQSPSSLSASVGDRVTITCRASQSISTYLNWYQQKPGKAPKLLIYAASTLQSGVPSRFGGSGSGTDFTLTVSSLQPEDFATYYCQQSYSTPPITFGQGTRLEIN

SEQ ID NO: 213 - protein, 122 aa, synthetic construct
  REGION 1..122: note = synthetic construct; antigen binding domain
QVQLVQSGAEVKKPGASVKVSCKTSGYTFTNNGISWVRQVPGQGLEWMGWISPYNGNTKYAQKFQGRVTMTTDTSTTTVYMDVRSLRSDDTAVYFCARDGPITISYFGMDVWGQGTTVTVSS

SEQ ID NO: 214 - protein, 108 aa, synthetic construct
  REGION 1..108: note = synthetic construct; antigen binding domain
EIVLTQSPDTLSLSPGERATLSCRASQSVAGSYLAWYQQKPGQAPRLLIYGASSRATGIPDRFSGSGSGTDFTLTISRLEPEDFAVYYCQQYGTSPWTFGQGTKVEIT

SEQ ID NO: 215 - protein, 118 aa, synthetic construct
  REGION 1..118: note = synthetic construct; antigen binding domain
QVQLVESGGGVVQPGRSLRLSCAASGFTVNRYGIHWVRQAPGKGLEWVAVTWYDGRNKYFADSVKGRFSFSRDSSTNTLYLQMNSLRAEDTAVYYCARGGLFGYFDYWGQGTLVTVSS

SEQ ID NO: 216 - protein, 107 aa, synthetic construct
  REGION 1..107: note = synthetic construct; antigen binding domain
EIVLTQSPGTLSLSPGERATLSCRASQSVSSYLAWYQQKPGQAPRLLIYGASSRATGIPDRFSGSGSGTDFILTINRLEPEDFAVYYCQHYGNSPWTFGQGTKVEIK

SEQ ID NO: 217 - protein, 118 aa, synthetic construct
  REGION 1..118: note = synthetic construct; antigen binding domain
QVQLVESGGGVVQPGRSLRLSCAASGFTFSSYGIHWVRQAPGKGLEWVAVIWYGGNNKYYADSVKGRFTISRDNSKNTLYLQMNSLRAEDTALYHCARSGNFGAFDIWGQGTMVTVSS